European Patent Specification EP 3 527 588 B1, published January 15, 2025. Title: Anti-FcRn Antibodies. Applicant: UCB Biopharma SPRL. The sequence listing filed with the application follows.

SEQUENCE LISTING (95 sequences)

SEQ ID NO: 1 - protein, 10 aa, Artificial
  CA170_1519 CDRH1
GFTFSNYGMV

SEQ ID NO: 2 - protein, 17 aa, Artificial
  CA170_1519 CDRH2
YIDSDGDNTYYRDSVKG

SEQ ID NO: 3 - protein, 8 aa, Artificial
  CA170_1519 CDRH3
GIVRPFLY

SEQ ID NO: 4 - protein, 16 aa, Artificial
  CA170_1519 CDRL1
KSSQSLVGASGKTYLY

SEQ ID NO: 5 - protein, 7 aa, Artificial
  CA170_1519 CDRL2
LVSTLDS

SEQ ID NO: 6 - protein, 9 aa, Artificial
  CA170_1519 CDRL3
LQGTHFPHT

SEQ ID NO: 7 - protein, 112 aa, Artificial
  Rat Ab 1519 VL region
DVVMTQTPLSLSVALGQPASISCKSSQSLVGASGKTYLYWLFQRSGQSPKRLIYLVSTLDSGIPDRFSGSGAETDFTLKIRRVEADDLGVYYCLQGTHFPHTFGAGTKLELK

SEQ ID NO: 8 - DNA, 336 bp, Artificial
  Rat Ab 1519 VL region
gatgttgtgatgacccagactccactgtctttgtcggttgcccttggacaaccagcctccatctcttgcaagtcaagtcagagcctcgtaggtgctagtggaaagacatatttgtattggttatttcagaggtccggccagtctccaaagcgactaatctatctggtgtccacactggactctggaattcctgataggttcagtggcagtggagcagagacagattttactcttaaaatccgcagagtggaagccgatgatttgggagtttattactgcttgcaaggtacacattttcctcacacgtttggagctgggaccaagctggaattgaaa

SEQ ID NO: 9 - protein, 132 aa, Artificial
  Rat Ab 1519 VL region with signal sequence
MMSPAQFLFLLMLWIQGTSGDVVMTQTPLSLSVALGQPASISCKSSQSLVGASGKTYLYWLFQRSGQSPKRLIYLVSTLDSGIPDRFSGSGAETDFTLKIRRVEADDLGVYYCLQGTHFPHTFGAGTKLELK

SEQ ID NO: 10 - DNA, 396 bp, Artificial
  Rat Ab 1519 VL region with signal sequence
atgatgagtcctgcccagttcctgtttctgctgatgctctggattcagggaaccagtggtgatgttgtgatgacccagactccactgtctttgtcggttgcccttggacaaccagcctccatctcttgcaagtcaagtcagagcctcgtaggtgctagtggaaagacatatttgtattggttatttcagaggtccggccagtctccaaagcgactaatctatctggtgtccacactggactctggaattcctgataggttcagtggcagtggagcagagacagattttactcttaaaatccgcagagtggaagccgatgatttgggagtttattactgcttgcaaggtacacattttcctcacacgtttggagctgggaccaagctggaattgaaa

SEQ ID NO: 11 - protein, 116 aa, Artificial
  Rat Ab 1519 VH region
EVPLVESGGGSVQPGRSMKLSCVVSGFTFSNYGMVWVRQAPKKGLEWVAYIDSDGDNTYYRDSVKGRFTISRNNAKSTLYLQMDSLRSEDTATYYCTTGIVRPFLYWGQGTTVTVS

SEQ ID NO: 12 - DNA, 348 bp, Artificial
  Rat Ab 1519 VH region
gaggtgccgctggtggagtctgggggcggctcagtgcagcctgggaggtccatgaaactctcctgtgtagtctcaggattcactttcagtaattatggcatggtctgggtccgccaggctccaaagaagggtctggagtgggtcgcatatattgattctgatggtgataatacttactaccgagattccgtgaagggccgattcactatctccagaaataatgcaaaaagcaccctatatttgcaaatggacagtctgaggtctgaggacacggccacttattactgtacaacagggattgtccggccctttctctattggggccaaggaaccacggtcaccgtctcg

SEQ ID NO: 13 - protein, 135 aa, Artificial
  Rat Ab 1519 VH region with signal sequence
MDISLSLAFLVLFIKGVRCEVPLVESGGGSVQPGRSMKLSCVVSGFTFSNYGMVWVRQAPKKGLEWVAYIDSDGDNTYYRDSVKGRFTISRNNAKSTLYLQMDSLRSEDTATYYCTTGIVRPFLYWGQGTTVTVS

SEQ ID NO: 14 - DNA, 405 bp, Artificial
  Rat Ab 1519 VH region with signal sequence
atggacatcagtctcagcttggctttccttgtccttttcataaaaggtgtccggtgtgaggtgccgctggtggagtctgggggcggctcagtgcagcctgggaggtccatgaaactctcctgtgtagtctcaggattcactttcagtaattatggcatggtctgggtccgccaggctccaaagaagggtctggagtgggtcgcatatattgattctgatggtgataatacttactaccgagattccgtgaagggccgattcactatctccagaaataatgcaaaaagcaccctatatttgcaaatggacagtctgaggtctgaggacacggccacttattactgtacaacagggattgtccggccctttctctattggggccaaggaaccacggtcaccgtctcg

SEQ ID NO: 15 - protein, 112 aa, Artificial [sequence omitted]

SEQ ID NO: 16 - DNA, 336 bp, Artificial
  1519 gL20 V-region (E. coli expression)
gatatccagatgacccagagtccaagcagtctctccgccagcgtaggcgatcgtgtgactattacctgtaaaagctcccagtccctggtgggtgcaagcggcaaaacctacctgtactggctcttccagaaaccgggcaaagctccgaaacgcctgatctatctggtgtctaccctggatagcggtattccgtctcgtttctccggtagcggtagcggtaccgaattcacgctgaccattagctccctccagccggaggactttgctacctattactgcctccagggcactcattttccgcacactttcggccagggtaccaaactggaaatcaaa

SEQ ID NO: 17 - DNA, 336 bp, Artificial
  1519 gL20 V-region (mammalian expression)
gatatccagatgacccagagcccatctagcttatccgcttccgttggtgatcgcgtgacaattacgtgtaagagctcccaatctctcgtgggtgcaagtggcaagacctatctgtactggctctttcagaagcctggcaaggcaccaaaacggctgatctatctggtgtctacccttgactctgggataccgtcacgattttccggatctgggagcggaactgagttcacactcacgatttcatcgctgcaacccgaggactttgctacctactactgcctgcaaggcactcatttccctcacactttcggccaggggacaaaactcgaaatcaaa

SEQ ID NO: 18 - protein, 133 aa, Artificial
  1519 gL20 V-region with signal sequence (E. coli expression)
MKKTAIAIAVALAGFATVAQADIQMTQSPSSLSASVGDRVTITCKSSQSLVGASGKTYLYWLFQKPGKAPKRLIYLVSTLDSGIPSRFSGSGSGTEFTLTISSLQPEDFATYYCLQGTHFPHTFGQGTKLEIK

SEQ ID NO: 19 - DNA, 399 bp, Artificial
  1519 gL20 V-region with signal sequence (E. coli expression)
atgaaaaagacagctatcgcaattgcagtggccttggctggtttcgctaccgtagcgcaagctgatatccagatgacccagagtccaagcagtctctccgccagcgtaggcgatcgtgtgactattacctgtaaaagctcccagtccctggtgggtgcaagcggcaaaacctacctgtactggctcttccagaaaccgggcaaagctccgaaacgcctgatctatctggtgtctaccctggatagcggtattccgtctcgtttctccggtagcggtagcggtaccgaattcacgctgaccattagctccctccagccggaggactttgctacctattactgcctccagggcactcattttccgcacactttcggccagggtaccaaactggaaatcaaa

SEQ ID NO: 20 - protein, 132 aa, Artificial
  1519 gL20 V-region with signal sequence (mammalian expression)
MSVPTQVLGLLLLWLTDARCDIQMTQSPSSLSASVGDRVTITCKSSQSLVGASGKTYLYWLFQKPGKAPKRLIYLVSTLDSGIPSRFSGSGSGTEFTLTISSLQPEDFATYYCLQGTHFPHTFGQGTKLEIK

SEQ ID NO: 21 - DNA, 396 bp, Artificial
  1519 gL20 V-region with signal sequence (mammalian expression)
atgtctgtccccacccaagtcctcggactcctgctactctggcttacagatgccagatgcgatatccagatgacccagagcccatctagcttatccgcttccgttggtgatcgcgtgacaattacgtgtaagagctcccaatctctcgtgggtgcaagtggcaagacctatctgtactggctctttcagaagcctggcaaggcaccaaaacggctgatctatctggtgtctacccttgactctgggataccgtcacgattttccggatctgggagcggaactgagttcacactcacgatttcatcgctgcaacccgaggactttgctacctactactgcctgcaaggcactcatttccctcacactttcggccaggggacaaaactcgaaatcaaa

SEQ ID NO: 22 - protein, 219 aa, Artificial
  1519 gL20 light chain (V + constant)
DIQMTQSPSSLSASVGDRVTITCKSSQSLVGASGKTYLYWLFQKPGKAPKRLIYLVSTLDSGIPSRFSGSGSGTEFTLTISSLQPEDFATYYCLQGTHFPHTFGQGTKLEIKRTVAAPSVFIFPPSDEQLKSGTASVVCLLNNFYPREAKVQWKVDNALQSGNSQESVTEQDSKDSTYSLSSTLTLSKADYEKHKVYACEVTHQGLSSPVTKSFNRGEC

SEQ ID NO: 23 - DNA, 657 bp, Artificial
  1519 gL20 light chain (V + constant, E. coli expression)
gatatccagatgacccagagtccaagcagtctctccgccagcgtaggcgatcgtgtgactattacctgtaaaagctcccagtccctggtgggtgcaagcggcaaaacctacctgtactggctcttccagaaaccgggcaaagctccgaaacgcctgatctatctggtgtctaccctggatagcggtattccgtctcgtttctccggtagcggtagcggtaccgaattcacgctgaccattagctccctccagccggaggactttgctacctattactgcctccagggcactcattttccgcacactttcggccagggtaccaaactggaaatcaaacgtacggtagcggccccatctgtcttcatcttcccgccatctgatgagcagttgaaatctggaactgcctctgttgtgtgcctgctgaataacttctatcccagagaggccaaagtacagtggaaggtggataacgccctccaatcgggtaactcccaggagagtgtcacagagcaggacagcaaggacagcacctacagcctcagcagcaccctgacgctgagcaaagcagactacgagaaacacaaagtctacgcctgcgaagtcacccatcagggcctgagctcaccagtaacaaaaagttttaatagaggggagtgt

SEQ ID NO: 24 - DNA, 657 bp, Artificial
  1519 gL20 light chain (V + constant, mammalian expression)
gatatccagatgacccagagtccaagcagtctctccgccagcgtaggcgatcgtgtgactattacctgtaaaagctcccagtccctggtgggtgcaagcggcaaaacctacctgtactggctcttccagaaaccgggcaaagctccgaaacgcctgatctatctggtgtctaccctggatagcggtattccgtctcgtttctccggtagcggtagcggtaccgaattcacgctgaccattagctccctccagccggaggactttgctacctattactgcctccagggcactcattttccgcacactttcggccagggtaccaaactggaaatcaaacgtacggtagcggccccatctgtcttcatcttcccgccatctgatgagcagttgaaatctggaactgcctctgttgtgtgcctgctgaataacttctatcccagagaggccaaagtacagtggaaggtggataacgccctccaatcgggtaactcccaggagagtgtcacagagcaggacagcaaggacagcacctacagcctcagcagcaccctgacgctgagcaaagcagactacgagaaacacaaagtctacgcctgcgaagtcacccatcagggcctgagctcgcccgtcacaaagagcttcaacaggggagagtgt

SEQ ID NO: 25 - protein, 240 aa, Artificial
  1519 gL20 light chain with signal sequence (E. coli expression)
MKKTAIAIAVALAGFATVAQADIQMTQSPSSLSASVGDRVTITCKSSQSLVGASGKTYLYWLFQKPGKAPKRLIYLVSTLDSGIPSRFSGSGSGTEFTLTISSLQPEDFATYYCLQGTHFPHTFGQGTKLEIKRTVAAPSVFIFPPSDEQLKSGTASVVCLLNNFYPREAKVQWKVDNALQSGNSQESVTEQDSKDSTYSLSSTLTLSKADYEKHKVYACEVTHQGLSSPVTKSFNRGEC

SEQ ID NO: 26 - DNA, 720 bp, Artificial
  1519 gL20 light chain with signal sequence (E. coli expression)
atgaaaaagacagctatcgcaattgcagtggccttggctggtttcgctaccgtagcgcaagctgatatccagatgacccagagtccaagcagtctctccgccagcgtaggcgatcgtgtgactattacctgtaaaagctcccagtccctggtgggtgcaagcggcaaaacctacctgtactggctcttccagaaaccgggcaaagctccgaaacgcctgatctatctggtgtctaccctggatagcggtattccgtctcgtttctccggtagcggtagcggtaccgaattcacgctgaccattagctccctccagccggaggactttgctacctattactgcctccagggcactcattttccgcacactttcggccagggtaccaaactggaaatcaaacgtacggtagcggccccatctgtcttcatcttcccgccatctgatgagcagttgaaatctggaactgcctctgttgtgtgcctgctgaataacttctatcccagagaggccaaagtacagtggaaggtggataacgccctccaatcgggtaactcccaggagagtgtcacagagcaggacagcaaggacagcacctacagcctcagcagcaccctgacgctgagcaaagcagactacgagaaacacaaagtctacgcctgcgaagtcacccatcagggcctgagctcaccagtaacaaaaagttttaatagaggggagtgt

SEQ ID NO: 27 - protein, 239 aa, Artificial
  1519 gL20 light chain with signal sequence (mammalian expression)
MSVPTQVLGLLLLWLTDARCDIQMTQSPSSLSASVGDRVTITCKSSQSLVGASGKTYLYWLFQKPGKAPKRLIYLVSTLDSGIPSRFSGSGSGTEFTLTISSLQPEDFATYYCLQGTHFPHTFGQGTKLEIKRTVAAPSVFIFPPSDEQLKSGTASVVCLLNNFYPREAKVQWKVDNALQSGNSQESVTEQDSKDSTYSLSSTLTLSKADYEKHKVYACEVTHQGLSSPVTKSFNRGEC

SEQ ID NO: 28 - DNA, 717 bp, Artificial
  1519 gL20 light chain with signal sequence (mammalian expression)
atgtctgtccccacccaagtcctcggactcctgctactctggcttacagatgccagatgcgatatccagatgacccagagcccatctagcttatccgcttccgttggtgatcgcgtgacaattacgtgtaagagctcccaatctctcgtgggtgcaagtggcaagacctatctgtactggctctttcagaagcctggcaaggcaccaaaacggctgatctatctggtgtctacccttgactctgggataccgtcacgattttccggatctgggagcggaactgagttcacactcacgatttcatcgctgcaacccgaggactttgctacctactactgcctgcaaggcactcatttccctcacactttcggccaggggacaaaactcgaaatcaaacgtacggtagcggccccatctgtcttcatcttcccgccatctgatgagcagttgaaatctggaactgcctctgttgtgtgcctgctgaataacttctatcccagagaggccaaagtacagtggaaggtggataacgccctccaatcgggtaactcccaggagagtgtcacagagcaggacagcaaggacagcacctacagcctcagcagcaccctgacgctgagcaaagcagactacgagaaacacaaagtctacgcctgcgaagtcacccatcagggcctgagctcgcccgtcacaaagagcttcaacaggggagagtgt

SEQ ID NO: 29 - protein, 116 aa, Artificial
  1519 gH20 V-region
EVPLVESGGGLVQPGGSLRLSCAVSGFTFSNYGMVWVRQAPGKGLEWVAYIDSDGDNTYYRDSVKGRFTISRDNAKSSLYLQMNSLRAEDTAVYYCTTGIVRPFLYWGQGTLVTVS

SEQ ID NO: 30 - DNA, 348 bp, Artificial
  1519 gH20 V-region (E. coli expression)
gaggttccgctggtcgagtctggaggcgggcttgtccagcctggagggagcctgcgtctctcttgtgcagtatctggcttcacgttctccaactacggtatggtgtgggttcgtcaggctccaggtaaaggtctggaatgggtggcgtatattgactccgacggcgacaacacctactatcgcgactctgtgaaaggtcgcttcaccatttcccgcgataacgccaaatccagcctgtacctgcagatgaacagcctgcgtgctgaagatactgcggtgtactattgcaccactggcatcgtgcgtccgtttctgtattggggtcagggtaccctcgttactgtctcg

SEQ ID NO: 31 - DNA, 348 bp, Artificial
  1519 gH20 V-region (mammalian expression)
gaggtaccacttgtggaaagcggaggaggtcttgtgcagcctggaggaagtttacgtctctcttgtgctgtgtctggcttcaccttctccaattacggaatggtctgggtcagacaagcacctggaaagggtcttgaatgggtggcctatattgactctgacggggacaacacctactatcgggattccgtgaaaggacgcttcacaatctcccgagataacgccaagagctcactgtacctgcagatgaatagcctgagagccgaggatactgccgtgtactattgcacaacgggaatcgttaggccttttctgtactggggacagggcaccttggttactgtctcg

SEQ ID NO: 32 - protein, 137 aa, Artificial
  1519 gH20 V-region (E. coli expression)
MKKTAIAIAVALAGFATVAQAEVPLVESGGGLVQPGGSLRLSCAVSGFTFSNYGMVWVRQAPGKGLEWVAYIDSDGDNTYYRDSVKGRFTISRDNAKSSLYLQMNSLRAEDTAVYYCTTGIVRPFLYWGQGTLVTVS

SEQ ID NO: 33 - DNA, 411 bp, Artificial
  1519 gH20 V-region (E. coli expression)
atgaagaagactgctatagcaattgcagtggcgctagctggtttcgccaccgtggcgcaagctgaggttccgctggtcgagtctggaggcgggcttgtccagcctggagggagcctgcgtctctcttgtgcagtatctggcttcacgttctccaactacggtatggtgtgggttcgtcaggctccaggtaaaggtctggaatgggtggcgtatattgactccgacggcgacaacacctactatcgcgactctgtgaaaggtcgcttcaccatttcccgcgataacgccaaatccagcctgtacctgcagatgaacagcctgcgtgctgaagatactgcggtgtactattgcaccactggcatcgtgcgtccgtttctgtattggggtcagggtaccctcgttactgtctcg

SEQ ID NO: 34 - protein, 135 aa, Artificial
  1519 gH20 V-region (mammalian expression)
MEWSWVFLFFLSVTTGVHSEVPLVESGGGLVQPGGSLRLSCAVSGFTFSNYGMVWVRQAPGKGLEWVAYIDSDGDNTYYRDSVKGRFTISRDNAKSSLYLQMNSLRAEDTAVYYCTTGIVRPFLYWGQGTLVTVS

SEQ ID NO: 35 - DNA, 405 bp, Artificial
  1519 gH20 V-region with signal sequence (mammalian expression)
atggaatggagctgggtctttctcttcttcctgtcagtaactacaggagtccattctgaggtaccacttgtggaaagcggaggaggtcttgtgcagcctggaggaagtttacgtctctcttgtgctgtgtctggcttcaccttctccaattacggaatggtctgggtcagacaagcacctggaaagggtcttgaatgggtggcctatattgactctgacggggacaacacctactatcgggattccgtgaaaggacgcttcacaatctcccgagataacgccaagagctcactgtacctgcagatgaatagcctgagagccgaggatactgccgtgtactattgcacaacgggaatcgttaggccttttctgtactggggacagggcaccttggttactgtctcg

SEQ ID NO: 36 - protein, 228 aa, Artificial
  1519gH20 Fab' heavy chain (V + human gamma-1 CH1 + hinge)
EVPLVESGGGLVQPGGSLRLSCAVSGFTFSNYGMVWVRQAPGKGLEWVAYIDSDGDNTYYRDSVKGRFTISRDNAKSSLYLQMNSLRAEDTAVYYCTTGIVRPFLYWGQGTLVTVSSASTKGPSVFPLAPSSKSTSGGTAALGCLVKDYFPEPVTVSWNSGALTSGVHTFPAVLQSSGLYSLSSVVTVPSSSLGTQTYICNVNHKPSNTKVDKKVEPKSCDKTHTCAA

SEQ ID NO: 37 - DNA, 684 bp, Artificial
  1519gH20 Fab' heavy chain (V + human gamma-1 CH1 + hinge, E.coli expression)
gaggttccgctggtcgagtctggaggcgggcttgtccagcctggagggagcctgcgtctctcttgtgcagtatctggcttcacgttctccaactacggtatggtgtgggttcgtcaggctccaggtaaaggtctggaatgggtggcgtatattgactccgacggcgacaacacctactatcgcgactctgtgaaaggtcgcttcaccatttcccgcgataacgccaaatccagcctgtacctgcagatgaacagcctgcgtgctgaagatactgcggtgtactattgcaccactggcatcgtgcgtccgtttctgtattggggtcagggtaccctcgttactgtctcgagcgcttctacaaagggcccatcggtcttccccctggcaccctcctccaagagcacctctgggggcacagcggccctgggctgcctggtcaaggactacttccccgaaccggtgacggtgtcgtggaactcaggcgccctgaccagcggcgtgcacaccttcccggctgtcctacagtcctcaggactctactccctcagcagcgtggtgaccgtgccctccagcagcttgggcacccagacctacatctgcaacgtgaatcacaagcccagcaacaccaaggtcgacaagaaagttgagcccaaatcttgtgacaaaactcacacatgcgccgcg

SEQ ID NO: 38 - DNA, 684 bp, Artificial
  1519gH20 Fab' heavy chain (V + human gamma-1 CH1 + hinge, mammalian expression)
gaggtaccacttgtggaaagcggaggaggtcttgtgcagcctggaggaagtttacgtctctcttgtgctgtgtctggcttcaccttctccaattacggaatggtctgggtcagacaagcacctggaaagggtcttgaatgggtggcctatattgactctgacggggacaacacctactatcgggattccgtgaaaggacgcttcacaatctcccgagataacgccaagagctcactgtacctgcagatgaatagcctgagagccgaggatactgccgtgtactattgcacaacgggaatcgttaggccttttctgtactggggacagggcaccttggttactgtctcgagcgcttctacaaagggcccatcggtcttccccctggcaccctcctccaagagcacctctgggggcacagcggccctgggctgcctggtcaaggactacttccccgaaccggtgacggtgtcgtggaactcaggcgccctgaccagcggcgtgcacaccttcccggctgtcctacagtcctcaggactctactccctcagcagcgtggtgaccgtgccctccagcagcttgggcacccagacctacatctgcaacgtgaatcacaagcccagcaacaccaaggtcgacaagaaagttgagcccaaatcttgtgacaaaactcacacatgcgccgcg

SEQ ID NO: 39 - protein, 249 aa, Artificial
  1519 gH20 Fab' heavy chain with signal sequence (E. coli expression)
MKKTAIAIAVALAGFATVAQAEVPLVESGGGLVQPGGSLRLSCAVSGFTFSNYGMVWVRQAPGKGLEWVAYIDSDGDNTYYRDSVKGRFTISRDNAKSSLYLQMNSLRAEDTAVYYCTTGIVRPFLYWGQGTLVTVSSASTKGPSVFPLAPSSKSTSGGTAALGCLVKDYFPEPVTVSWNSGALTSGVHTFPAVLQSSGLYSLSSVVTVPSSSLGTQTYICNVNHKPSNTKVDKKVEPKSCDKTHTCAA

SEQ ID NO: 40 - DNA, 747 bp, Artificial
  1519 gH20 Fab' heavy chain with signal sequence (E. coli expression)
atgaagaagactgctatagcaattgcagtggcgctagctggtttcgccaccgtggcgcaagctgaggttccgctggtcgagtctggaggcgggcttgtccagcctggagggagcctgcgtctctcttgtgcagtatctggcttcacgttctccaactacggtatggtgtgggttcgtcaggctccaggtaaaggtctggaatgggtggcgtatattgactccgacggcgacaacacctactatcgcgactctgtgaaaggtcgcttcaccatttcccgcgataacgccaaatccagcctgtacctgcagatgaacagcctgcgtgctgaagatactgcggtgtactattgcaccactggcatcgtgcgtccgtttctgtattggggtcagggtaccctcgttactgtctcgagcgcttctacaaagggcccatcggtcttccccctggcaccctcctccaagagcacctctgggggcacagcggccctgggctgcctggtcaaggactacttccccgaaccggtgacggtgtcgtggaactcaggcgccctgaccagcggcgtgcacaccttcccggctgtcctacagtcctcaggactctactccctcagcagcgtggtgaccgtgccctccagcagcttgggcacccagacctacatctgcaacgtgaatcacaagcccagcaacaccaaggtcgacaagaaagttgagcccaaatcttgtgacaaaactcacacatgcgccgcg

SEQ ID NO: 41 - protein, 247 aa, Artificial
  1519 gH20 Fab' heavy chain with signal sequence (mammalian expression)
MEWSWVFLFFLSVTTGVHSEVPLVESGGGLVQPGGSLRLSCAVSGFTFSNYGMVWVRQAPGKGLEWVAYIDSDGDNTYYRDSVKGRFTISRDNAKSSLYLQMNSLRAEDTAVYYCTTGIVRPFLYWGQGTLVTVSSASTKGPSVFPLAPSSKSTSGGTAALGCLVKDYFPEPVTVSWNSGALTSGVHTFPAVLQSSGLYSLSSVVTVPSSSLGTQTYICNVNHKPSNTKVDKKVEPKSCDKTHTCAA

SEQ ID NO: 42 - DNA, 741 bp, Artificial
  1519 gH20 Fab' heavy chain with signal sequence (mammalian expression)
atggaatggagctgggtctttctcttcttcctgtcagtaactacaggagtccattctgaggtaccacttgtggaaagcggaggaggtcttgtgcagcctggaggaagtttacgtctctcttgtgctgtgtctggcttcaccttctccaattacggaatggtctgggtcagacaagcacctggaaagggtcttgaatgggtggcctatattgactctgacggggacaacacctactatcgggattccgtgaaaggacgcttcacaatctcccgagataacgccaagagctcactgtacctgcagatgaatagcctgagagccgaggatactgccgtgtactattgcacaacgggaatcgttaggccttttctgtactggggacagggcaccttggttactgtctcgagcgcttctacaaagggcccatcggtcttccccctggcaccctcctccaagagcacctctgggggcacagcggccctgggctgcctggtcaaggactacttccccgaaccggtgacggtgtcgtggaactcaggcgccctgaccagcggcgtgcacaccttcccggctgtcctacagtcctcaggactctactccctcagcagcgtggtgaccgtgccctccagcagcttgggcacccagacctacatctgcaacgtgaatcacaagcccagcaacaccaaggtcgacaagaaagttgagcccaaatcttgtgacaaaactcacacatgcgccgcg

SEQ ID NO: 43 - protein, 444 aa, Artificial
  1519gH20 IgG4 heavy chain (V + human gamma-4P constant)
EVPLVESGGGLVQPGGSLRLSCAVSGFTFSNYGMVWVRQAPGKGLEWVAYIDSDGDNTYYRDSVKGRFTISRDNAKSSLYLQMNSLRAEDTAVYYCTTGIVRPFLYWGQGTLVTVSSASTKGPSVFPLAPCSRSTSESTAALGCLVKDYFPEPVTVSWNSGALTSGVHTFPAVLQSSGLYSLSSVVTVPSSSLGTKTYTCNVDHKPSNTKVDKRVESKYGPPCPPCPAPEFLGGPSVFLFPPKPKDTLMISRTPEVTCVVVDVSQEDPEVQFNWYVDGVEVHNAKTKPREEQFNSTYRVVSVLTVLHQDWLNGKEYKCKVSNKGLPSSIEKTISKAKGQPREPQVYTLPPSQEEMTKNQVSLTCLVKGFYPSDIAVEWESNGQPENNYKTTPPVLDSDGSFFLYSRLTVDKSRWQEGNVFSCSVMHEALHNHYTQKSLSLSLGK

SEQ ID NO: 44 - DNA, 1939 bp, Artificial
  1519gH20 IgG4 heavy chain (V + human gamma-4P constant with exons)
gaggtaccacttgtggaaagcggaggaggtcttgtgcagcctggaggaagtttacgtctctcttgtgctgtgtctggcttcaccttctccaattacggaatggtctgggtcagacaagcacctggaaagggtcttgaatgggtggcctatattgactctgacggggacaacacctactatcgggattccgtgaaaggacgcttcacaatctcccgagataacgccaagagctcactgtacctgcagatgaatagcctgagagccgaggatactgccgtgtactattgcacaacgggaatcgttaggccttttctgtactggggacagggcaccttggttactgtctcgagcgcttctacaaagggcccatccgtcttccccctggcgccctgctccaggagcacctccgagagcacagccgccctgggctgcctggtcaaggactacttccccgaaccggtgacggtgtcgtggaactcaggcgccctgaccagcggcgtgcacaccttcccggctgtcctacagtcctcaggactctactccctcagcagcgtggtgaccgtgccctccagcagcttgggcacgaagacctacacctgcaacgtagatcacaagcccagcaacaccaaggtggacaagagagttggtgagaggccagcacagggagggagggtgtctgctggaagccaggctcagccctcctgcctggacgcaccccggctgtgcagccccagcccagggcagcaaggcatgccccatctgtctcctcacccggaggcctctgaccaccccactcatgcccagggagagggtcttctggatttttccaccaggctccgggcagccacaggctggatgcccctaccccaggccctgcgcatacaggggcaggtgctgcgctcagacctgccaagagccatatccgggaggaccctgcccctgacctaagcccaccccaaaggccaaactctccactccctcagctcagacaccttctctcctcccagatctgagtaactcccaatcttctctctgcagagtccaaatatggtcccccatgcccaccatgcccaggtaagccaacccaggcctcgccctccagctcaaggcgggacaggtgccctagagtagcctgcatccagggacaggccccagccgggtgctgacgcatccacctccatctcttcctcagcacctgagttcctggggggaccatcagtcttcctgttccccccaaaacccaaggacactctcatgatctcccggacccctgaggtcacgtgcgtggtggtggacgtgagccaggaagaccccgaggtccagttcaactggtacgtggatggcgtggaggtgcataatgccaagacaaagccgcgggaggagcagttcaacagcacgtaccgtgtggtcagcgtcctcaccgtcctgcaccaggactggctgaacggcaaggagtacaagtgcaaggtctccaacaaaggcctcccgtcctccatcgagaaaaccatctccaaagccaaaggtgggacccacggggtgcgagggccacatggacagaggtcagctcggcccaccctctgccctgggagtgaccgctgtgccaacctctgtccctacagggcagccccgagagccacaggtgtacaccctgcccccatcccaggaggagatgaccaagaaccaggtcagcctgacctgcctggtcaaaggcttctaccccagcgacatcgccgtggagtgggagagcaatgggcagccggagaacaactacaagaccacgcctcccgtgctggactccgacggctccttcttcctctacagcaggctaaccgtggacaagagcaggtggcaggaggggaatgtcttctcatgctccgtgatgcatgaggctctgcacaaccactacacacagaagagcctctccctgtctctgggtaaa

SEQ ID NO: 45 - DNA, 1996 bp, Artificial
  1519gH20 IgG4 heavy chain (V + human gamma-4P constant) with signal sequence
atggaatggagctgggtctttctcttcttcctgtcagtaactacaggagtccattctgaggtaccacttgtggaaagcggaggaggtcttgtgcagcctggaggaagtttacgtctctcttgtgctgtgtctggcttcaccttctccaattacggaatggtctgggtcagacaagcacctggaaagggtcttgaatgggtggcctatattgactctgacggggacaacacctactatcgggattccgtgaaaggacgcttcacaatctcccgagataacgccaagagctcactgtacctgcagatgaatagcctgagagccgaggatactgccgtgtactattgcacaacgggaatcgttaggccttttctgtactggggacagggcaccttggttactgtctcgagcgcttctacaaagggcccatccgtcttccccctggcgccctgctccaggagcacctccgagagcacagccgccctgggctgcctggtcaaggactacttccccgaaccggtgacggtgtcgtggaactcaggcgccctgaccagcggcgtgcacaccttcccggctgtcctacagtcctcaggactctactccctcagcagcgtggtgaccgtgccctccagcagcttgggcacgaagacctacacctgcaacgtagatcacaagcccagcaacaccaaggtggacaagagagttggtgagaggccagcacagggagggagggtgtctgctggaagccaggctcagccctcctgcctggacgcaccccggctgtgcagccccagcccagggcagcaaggcatgccccatctgtctcctcacccggaggcctctgaccaccccactcatgcccagggagagggtcttctggatttttccaccaggctccgggcagccacaggctggatgcccctaccccaggccctgcgcatacaggggcaggtgctgcgctcagacctgccaagagccatatccgggaggaccctgcccctgacctaagcccaccccaaaggccaaactctccactccctcagctcagacaccttctctcctcccagatctgagtaactcccaatcttctctctgcagagtccaaatatggtcccccatgcccaccatgcccaggtaagccaacccaggcctcgccctccagctcaaggcgggacaggtgccctagagtagcctgcatccagggacaggccccagccgggtgctgacgcatccacctccatctcttcctcagcacctgagttcctggggggaccatcagtcttcctgttccccccaaaacccaaggacactctcatgatctcccggacccctgaggtcacgtgcgtggtggtggacgtgagccaggaagaccccgaggtccagttcaactggtacgtggatggcgtggaggtgcataatgccaagacaaagccgcgggaggagcagttcaacagcacgtaccgtgtggtcagcgtcctcaccgtcctgcaccaggactggctgaacggcaaggagtacaagtgcaaggtctccaacaaaggcctcccgtcctccatcgagaaaaccatctccaaagccaaaggtgggacccacggggtgcgagggccacatggacagaggtcagctcggcccaccctctgccctgggagtgaccgctgtgccaacctctgtccctacagggcagccccgagagccacaggtgtacaccctgcccccatcccaggaggagatgaccaagaaccaggtcagcctgacctgcctggtcaaaggcttctaccccagcgacatcgccgtggagtgggagagcaatgggcagccggagaacaactacaagaccacgcctcccgtgctggactccgacggctccttcttcctctacagcaggctaaccgtggacaagagcaggtggcaggaggggaatgtcttctcatgctccgtgatgcatgaggctctgcacaaccactacacacagaagagcctctccctgtctctgggtaaa

SEQ ID NO: 46 - protein, 347 aa, Artificial
  1519gL20 FabFv light chain
DIQMTQSPSSLSASVGDRVTITCKSSQSLVGASGKTYLYWLFQKPGKAPKRLIYLVSTLDSGIPSRFSGSGSGTEFTLTISSLQPEDFATYYCLQGTHFPHTFGQGTKLEIKRTVAAPSVFIFPPSDEQLKSGTASVVCLLNNFYPREAKVQWKVDNALQSGNSQESVTEQDSKDSTYSLSSTLTLSKADYEKHKVYACEVTHQGLSSPVTKSFNRGECSGGGGSGGGGSGGGGSDIQMTQSPSSVSASVGDRVTITCQSSPSVWSNFLSWYQQKPGKAPKLLIYEASKLTSGVPSRFSGSGSGTDFTLTISSLQPEDFATYYCGGGYSSISDTTFGCGTKVEIKRT

SEQ ID NO: 47 - DNA, 1041 bp, Artificial
  1519gL20 FabFv light chain
gatatccagatgacccagagcccatctagcttatccgcttccgttggtgatcgcgtgacaattacgtgtaagagctcccaatctctcgtgggtgcaagtggcaagacctatctgtactggctctttcagaagcctggcaaggcaccaaaacggctgatctatctggtgtctacccttgactctgggataccgtcacgattttccggatctgggagcggaactgagttcacactcacgatttcatcgctgcaacccgaggactttgctacctactactgcctgcaaggcactcatttccctcacactttcggccaggggacaaaactcgaaatcaaacgtacggtagcggccccatctgtcttcatcttcccgccatctgatgagcagttgaaatctggaactgcctctgttgtgtgcctgctgaataacttctatcccagagaggccaaagtacagtggaaggtggataacgccctccaatcgggtaactcccaggagagtgtcacagagcaggacagcaaggacagcacctacagcctgagcagcaccctgacgctgtctaaagcagactacgagaaacacaaagtgtacgcctgcgaagtcacccatcagggcctgagctcaccagtaacaaaaagttttaatagaggggagtgtagcggtggcggtggcagtggtgggggaggctccggaggtggcggttcagacatacaaatgacccagagtccttcatcggtatccgcgtccgttggcgatagggtgactattacatgtcaaagctctcctagcgtctggagcaattttctatcctggtatcaacagaaaccggggaaggctccaaaacttctgatttatgaagcctcgaaactcaccagtggagttccgtcaagattcagtggctctggatcagggacagacttcacgttgacaatcagttcgctgcaaccagaggactttgcgacctactattgtggtggaggttacagtagcataagtgatacgacatttgggtgcggtactaaggtggaaatcaaacgtacc

SEQ ID NO: 48 - protein, 367 aa, Artificial
  1519gL20 FabFv light chain with signal sequence
MSVPTQVLGLLLLWLTDARCDIQMTQSPSSLSASVGDRVTITCKSSQSLVGASGKTYLYWLFQKPGKAPKRLIYLVSTLDSGIPSRFSGSGSGTEFTLTISSLQPEDFATYYCLQGTHFPHTFGQGTKLEIKRTVAAPSVFIFPPSDEQLKSGTASVVCLLNNFYPREAKVQWKVDNALQSGNSQESVTEQDSKDSTYSLSSTLTLSKADYEKHKVYACEVTHQGLSSPVTKSFNRGECSGGGGSGGGGSGGGGSDIQMTQSPSSVSASVGDRVTITCQSSPSVWSNFLSWYQQKPGKAPKLLIYEASKLTSGVPSRFSGSGSGTDFTLTISSLQPEDFATYYCGGGYSSISDTTFGCGTKVEIKRT

SEQ ID NO: 49 - DNA, 1101 bp, Artificial
  1519gL20 FabFv light chain with signal sequence
atgtctgtccccacccaagtcctcggactcctgctactctggcttacagatgccagatgcgatatccagatgacccagagcccatctagcttatccgcttccgttggtgatcgcgtgacaattacgtgtaagagctcccaatctctcgtgggtgcaagtggcaagacctatctgtactggctctttcagaagcctggcaaggcaccaaaacggctgatctatctggtgtctacccttgactctgggataccgtcacgattttccggatctgggagcggaactgagttcacactcacgatttcatcgctgcaacccgaggactttgctacctactactgcctgcaaggcactcatttccctcacactttcggccaggggacaaaactcgaaatcaaacgtacggtagcggccccatctgtcttcatcttcccgccatctgatgagcagttgaaatctggaactgcctctgttgtgtgcctgctgaataacttctatcccagagaggccaaagtacagtggaaggtggataacgccctccaatcgggtaactcccaggagagtgtcacagagcaggacagcaaggacagcacctacagcctgagcagcaccctgacgctgtctaaagcagactacgagaaacacaaagtgtacgcctgcgaagtcacccatcagggcctgagctcaccagtaacaaaaagttttaatagaggggagtgtagcggtggcggtggcagtggtgggggaggctccggaggtggcggttcagacatacaaatgacccagagtccttcatcggtatccgcgtccgttggcgatagggtgactattacatgtcaaagctctcctagcgtctggagcaattttctatcctggtatcaacagaaaccggggaaggctccaaaacttctgatttatgaagcctcgaaactcaccagtggagttccgtcaagattcagtggctctggatcagggacagacttcacgttgacaatcagttcgctgcaaccagaggactttgcgacctactattgtggtggaggttacagtagcataagtgatacgacatttgggtgcggtactaaggtggaaatcaaacgtacc

SEQ ID NO: 50 - protein, 357 aa, Artificial
  1519gH20 FabFv heavy chain
EVPLVESGGGLVQPGGSLRLSCAVSGFTFSNYGMVWVRQAPGKGLEWVAYIDSDGDNTYYRDSVKGRFTISRDNAKSSLYLQMNSLRAEDTAVYYCTTGIVRPFLYWGQGTLVTVSSASTKGPSVFPLAPSSKSTSGGTAALGCLVKDYFPEPVTVSWNSGALTSGVHTFPAVLQSSGLYSLSSVVTVPSSSLGTQTYICNVNHKPSNTKVDKKVEPKSCSGGGGSGGGGTGGGGSEVQLLESGGGLVQPGGSLRLSCAVSGIDLSNYAINWVRQAPGKCLEWIGIIWASGTTFYATWAKGRFTISRDNSKNTVYLQMNSLRAEDTAVYYCARTVPGYSTAPYFDLWGQGTLVTVSS

SEQ ID NO: 51 - DNA, 1071 bp, Artificial
  1519gH20 FabFv heavy chain
gaggtaccacttgtggaaagcggaggaggtcttgtgcagcctggaggaagtttacgtctctcttgtgctgtgtctggcttcaccttctccaattacggaatggtctgggtcagacaagcacctggaaagggtcttgaatgggtggcctatattgactctgacggggacaacacctactatcgggattccgtgaaaggacgcttcacaatctcccgagataacgccaagagctcactgtacctgcagatgaatagcctgagagccgaggatactgccgtgtactattgcacaacgggaatcgttaggccttttctgtactggggacagggcaccttggttactgtctcgagcgcgtccacaaagggcccatcggtcttccccctggcaccctcctccaagagcacctctgggggcacagcggccctgggctgcctggtcaaggactacttccccgaaccagtgacggtgtcgtggaactcaggtgccctgaccagcggcgttcacaccttcccggctgtcctacagtcttcaggactctactccctgagcagcgtggtgaccgtgccctccagcagcttgggcacccagacctacatctgcaacgtgaatcacaagcccagcaacaccaaggtcgataagaaagttgagcccaaatcttgtagtggaggtgggggctcaggtggaggcgggaccggtggaggtggcagcgaggttcaactgcttgagtctggaggaggcctagtccagcctggagggagcctgcgtctctcttgtgcagtaagcggcatcgacctgagcaattacgccatcaactgggtgagacaagctccggggaagtgtttagaatggatcggtataatatgggccagtgggacgaccttttatgctacatgggcgaaaggaaggtttacaattagccgggacaatagcaaaaacaccgtgtatctccaaatgaactccttgcgagcagaggacacggcggtgtactattgtgctcgcactgtcccaggttatagcactgcaccctacttcgatctgtggggacaagggaccctggtgactgtttcaagt

SEQ ID NO: 52 - protein, 376 aa, Artificial
  1519gH20 FabFv heavy chain with signal sequence
MEWSWVFLFFLSVTTGVHSEVPLVESGGGLVQPGGSLRLSCAVSGFTFSNYGMVWVRQAPGKGLEWVAYIDSDGDNTYYRDSVKGRFTISRDNAKSSLYLQMNSLRAEDTAVYYCTTGIVRPFLYWGQGTLVTVSSASTKGPSVFPLAPSSKSTSGGTAALGCLVKDYFPEPVTVSWNSGALTSGVHTFPAVLQSSGLYSLSSVVTVPSSSLGTQTYICNVNHKPSNTKVDKKVEPKSCSGGGGSGGGGTGGGGSEVQLLESGGGLVQPGGSLRLSCAVSGIDLSNYAINWVRQAPGKCLEWIGIIWASGTTFYATWAKGRFTISRDNSKNTVYLQMNSLRAEDTAVYYCARTVPGYSTAPYFDLWGQGTLVTVSS

SEQ ID NO: 53 - DNA, 1128 bp, Artificial
  1519gH20 FabFv heavy chain with signal sequence
atggaatggagctgggtctttctcttcttcctgtcagtaactacaggagtccattctgaggtaccacttgtggaaagcggaggaggtcttgtgcagcctggaggaagtttacgtctctcttgtgctgtgtctggcttcaccttctccaattacggaatggtctgggtcagacaagcacctggaaagggtcttgaatgggtggcctatattgactctgacggggacaacacctactatcgggattccgtgaaaggacgcttcacaatctcccgagataacgccaagagctcactgtacctgcagatgaatagcctgagagccgaggatactgccgtgtactattgcacaacgggaatcgttaggccttttctgtactggggacagggcaccttggttactgtctcgagcgcgtccacaaagggcccatcggtcttccccctggcaccctcctccaagagcacctctgggggcacagcggccctgggctgcctggtcaaggactacttccccgaaccagtgacggtgtcgtggaactcaggtgccctgaccagcggcgttcacaccttcccggctgtcctacagtcttcaggactctactccctgagcagcgtggtgaccgtgccctccagcagcttgggcacccagacctacatctgcaacgtgaatcacaagcccagcaacaccaaggtcgataagaaagttgagcccaaatcttgtagtggaggtgggggctcaggtggaggcgggaccggtggaggtggcagcgaggttcaactgcttgagtctggaggaggcctagtccagcctggagggagcctgcgtctctcttgtgcagtaagcggcatcgacctgagcaattacgccatcaactgggtgagacaagctccggggaagtgtttagaatggatcggtataatatgggccagtgggacgaccttttatgctacatgggcgaaaggaaggtttacaattagccgggacaatagcaaaaacaccgtgtatctccaaatgaactccttgcgagcagaggacacggcggtgtactattgtgctcgcactgtcccaggttatagcactgcaccctacttcgatctgtggggacaagggaccctggtgactgtttcaagt

SEQ ID NO: 54 - protein, 107 aa, Artificial
  Human VK1 2-1-(1) A30 JK2 acceptor framework
DIQMTQSPSSLSASVGDRVTITCRASQGIRNDLGWYQQKPGKAPKRLIYAASSLQSGVPSRFSGSGSGTEFTLTISSLQPEDFATYYCLQHNSYPYTFGQGTKLEIK

SEQ ID NO: 55 - DNA, 321 bp, Artificial
  Human VK1 2-1-(1) A30 JK2 acceptor framework
gacatccagatgacccagtctccatcctccctgtctgcatctgtaggagacagagtcaccatcacttgccgggcaagtcagggcattagaaatgatttaggctggtatcagcagaaaccagggaaagcccctaagcgcctgatctatgctgcatccagtttgcaaagtggggtcccatcaaggttcagcggcagtggatctgggacagaattcactctcacaatcagcagcctgcagcctgaagattttgcaacttattactgtctacagcataatagttacccttacacttttggccaggggaccaagctggagatcaaa

SEQ ID NO: 56 - protein, 112 aa, Artificial
  Human VH3 1-3 3-07 JH4 acceptor framework
EVQLVESGGGLVQPGGSLRLSCAASGFTFSSYWMSWVRQAPGKGLEWVANIKQDGSEKYYVDSVKGRFTISRDNAKNSLYLQMNSLRAEDTAVYYCARYFDYWGQGTLVTVS

SEQ ID NO: 57 - DNA, 336 bp, Artificial
  Human VH3 1-3 3-07 JH4 acceptor framework
gaggtgcagctggtggagtctgggggaggcttggtccagcctggggggtccctgagactctcctgtgcagcctctggattcacctttagtagctattggatgagctgggtccgccaggctccagggaaggggctggagtgggtggccaacataaagcaagatggaagtgagaaatactatgtggactctgtgaagggccgattcaccatctccagagacaacgccaagaactcactgtatctgcaaatgaacagcctgagagccgaggacacggctgtgtattactgtgcgagatactttgactactggggccagggaaccctggtcaccgtctcc

SEQ ID NO: 58 - protein, 112 aa, Artificial
  Rat Ab 1548 VL region
DVVMTQTPLSLSVALGQPASISCKSSQSLVGASGKTYLYWLFQRSGQSPKRLIYLVSTLDSGIPDRFSGSGAETDFTLKIRRVEADDLGVYYCLQGTHFPHTFGAGTKLEIK

SEQ ID NO: 59 - DNA, 336 bp, Artificial
  Rat Ab 1548 VL region
gatgttgtgatgacccagactccactgtctttgtcggttgcccttggacaaccagcctccatctcttgcaagtcaagtcagagcctcgtaggtgctagtggaaagacatatttgtattggttatttcagaggtccggccagtctccaaagcgactaatctatctggtgtccacactggactctggaattcctgataggttcagtggcagtggagcagagacagattttactcttaaaatccgcagagtggaagccgatgatttgggagtttattactgcttgcaaggtacacattttcctcacacgtttggagctgggaccaagctggaaataaaa

SEQ ID NO: 60 - protein, 116 aa, Artificial
  Rat Ab 1548 VH region
EVPLVESGGGSVQPGRSMKLSCVVSGFTFSNYGMVWVRQAPKKGLEWVAYIDSDGDNTYYRDSVKGRFTISRNNAKSTLYLQMDSLRSEDTATYYCTTGIVRPFLYWGQGVMVTVS

SEQ ID NO: 61 - DNA, 348 bp, Artificial
  Rat Ab 1548 VH region
gaggtgccgctggtggagtctgggggcggctcagtgcagcctgggaggtccatgaaactctcctgtgtagtctcaggattcactttcagtaattatggcatggtctgggtccgccaggctccaaagaagggtctggagtgggtcgcatatattgattctgatggtgataatacttactaccgagattccgtgaagggccgattcactatctccagaaataatgcaaaaagcaccctatatttgcaaatggacagtctgaggtctgaggacacggccacttattactgtacaacagggattgtccggccctttctctattggggccaaggagtcatggtcacagtctcg

SEQ ID NO: 62 - protein, 112 aa, Artificial
  Rat Ab 1644 VL region
DVVMTQTPLSLSVAIGQPASISCKSSQSLVGASGKTYLYWLFQRSGQSPKRLIYLVSTLDSGIPDRFSGSGAETDFTLKIRRVEADDLGVYYCLQGTHFPHTFGAGTKLELK

SEQ ID NO: 63 - DNA, 336 bp, Artificial
  Rat Ab 1644 VL region
gatgttgtgatgacccagactccactgtctttgtcggttgccattggacaaccagcctccatctcttgcaagtcaagtcagagcctcgtaggtgctagtggaaagacatatttgtattggttatttcagaggtccggccagtctccaaagcgactaatctatctggtgtccacactggactctggaattcctgataggttcagtggcagtggagcagagacagattttactcttaaaatccgcagagtggaagccgatgatttgggagtttattactgcttgcaaggtacacattttcctcacacgtttggagctgggaccaagctggaactgaaa

SEQ ID NO: 64 - protein, 116 aa, Artificial
  Rat Ab 1644 VH region
EVPLVESGGGSVQPGRSTKLSCVVSGFTFSNYGMVWVRQAPKKGLEWVAYIGSDGDNIYYRDSVKGRFTISRNNAKSTLYLQMDSLRSEDTATYYCTTGIVRPFLYWGQGTTVTVS

SEQ ID NO: 65 - DNA, 348 bp, Artificial
  Rat Ab 1644 VH region
gaggtgccgctggtggagtctgggggcggctcagtgcagcctgggaggtccacgaaactctcctgtgtagtctcaggattcactttcagtaactatggcatggtctgggtccgccaggctccaaagaagggtctggagtgggtcgcatatattggttctgatggtgataatatttactaccgagattccgtgaagggtcgattcactatctccagaaataatgcaaaaagcaccctatatttgcaaatggacagtctgaggtctgaggacacggccacttattactgtacaacagggattgtccggccctttctctactggggccaaggaaccacggtcaccgtctcg

SEQ ID NO: 66 - protein, 112 aa, Artificial; identical to SEQ ID NO: 7
  Rat Ab 1496 VK region

SEQ ID NO: 67 - DNA, 336 bp, Artificial
  Rat Ab 1496 VK region
gatgttgtgatgacccagactccactgtctttgtcggttgcccttggacaaccagcctccatctcttgcaagtcaagtcagagcctcgtaggtgctagtggaaagacatatttgtattggttatttcagaggtccggccagtctccaaagcgactaatctatctggtgtccacactggactctggaattcctgataggttcagtggcagtggagcagagacagattttactcttaaaatccgcagagtggaagccgatgatttgggagtttattactgcttgcaaggtacacattttcctcacacgtttggagctgggaccaagctggaactgaaa

SEQ ID NO: 68 - protein, 116 aa, Artificial
  Rat Ab 1496 VH region
EVLLVESGGGSVQPGRSMKLSCVVSGFTFSNYGMVWVRQAPKKGLEWVAYIDSDGDNTYYRDSVKGRFTISRNNAKSTLYLQMDSLRSEDTATYYCTTGIVRPFLYWGQGTMVTVS

SEQ ID NO: 69 - DNA, 348 bp, Artificial
  Rat Ab 1496 VH region
gaggtgctgctggtggagtctgggggcggctcagtgcagcctgggaggtccatgaaactctcctgtgtagtctcaggattcactttcagtaattatggcatggtctgggtccgccaggctccaaagaagggtctggagtgggtcgcatatattgattctgatggtgataatacttactaccgagattccgtgaagggccgattcactatctccagaaataatgcaaaaagcaccctatatttgcaaatggacagtctgaggtctgaggacacggccacttattactgtacaacagggattgtccggccctttctctattggggccaaggaaccatggtcaccgtctcg

SEQ ID NO: 70 - protein, 14 aa, Artificial
  framework
YFDYWGQGTLVTVS

SEQ ID NO: 71 - protein, 12 aa, Artificial
  framework
YTFGQGTKLEIK

SEQ ID NO: 72 - protein, 447 aa, Artificial
  1519gH20 IgG1 heavy chain (V + human gamma-1 constant)
EVPLVESGGGLVQPGGSLRLSCAVSGFTFSNYGMVWVRQAPGKGLEWVAYIDSDGDNTYYRDSVKGRFTISRDNAKSSLYLQMNSLRAEDTAVYYCTTGIVRPFLYWGQGTLVTVSSASTKGPSVFPLAPSSKSTSGGTAALGCLVKDYFPEPVTVSWNSGALTSGVHTFPAVLQSSGLYSLSSVVTVPSSSLGTQTYICNVNHKPSNTKVDKKVEPKSCDKTHTCPPCPAPELLGGPSVFLFPPKPKDTLMISRTPEVTCVVVDVSHEDPEVKFNWYVDGVEVHNAKTKPREEQYNSTYRVVSVLTVLHQDWLNGKEYKCKVSNKALPAPIEKTISKAKGQPREPQVYTLPPSRDELTKNQVSLTCLVKGFYPSDIAVEWESNGQPENNYKTTPPVLDSDGSFFLYSKLTVDKSRWQQGNVFSCSVMHEALHNHYTQKSLSLSPGK

SEQ ID NO: 73 - DNA, 1947 bp, Artificial
  1519gH20 IgG1 heavy chain (V + human gamma-1 constant with exons)
gaggtaccacttgtggaaagcggaggaggtcttgtgcagcctggaggaagtttacgtctctcttgtgctgtgtctggcttcaccttctccaattacggaatggtctgggtcagacaagcacctggaaagggtcttgaatgggtggcctatattgactctgacggggacaacacctactatcgggattccgtgaaaggacgcttcacaatctcccgagataacgccaagagctcactgtacctgcagatgaatagcctgagagccgaggatactgccgtgtactattgcacaacgggaatcgttaggccttttctgtactggggacagggcaccttggttactgtctcgagcgcttctacaaagggcccatcggtcttccccctggcaccctcctccaagagcacctctgggggcacagcggccctgggctgcctggtcaaggactacttccccgaaccggtgacggtgtcgtggaactcaggcgccctgaccagcggcgtgcacaccttcccggctgtcctacagtcctcaggactctactccctcagcagcgtggtgaccgtgccctccagcagcttgggcacccagacctacatctgcaacgtgaatcacaagcccagcaacaccaaggtcgacaagaaagttggtgagaggccagcacagggagggagggtgtctgctggaagccaggctcagcgctcctgcctggacgcatcccggctatgcagccccagtccagggcagcaaggcaggccccgtctgcctcttcacccggaggcctctgcccgccccactcatgctcagggagagggtcttctggctttttccccaggctctgggcaggcacaggctaggtgcccctaacccaggccctgcacacaaaggggcaggtgctgggctcagacctgccaagagccatatccgggaggaccctgcccctgacctaagcccaccccaaaggccaaactctccactccctcagctcggacaccttctctcctcccagatctgagtaactcccaatcttctctctgcagagcccaaatcttgtgacaaaactcacacatgcccaccgtgcccaggtaagccagcccaggcctcgccctccagctcaaggcgggacaggtgccctagagtagcctgcatccagggacaggccccagccgggtgctgacacgtccacctccatctcttcctcagcacctgaactcctggggggaccgtcagtcttcctcttccccccaaaacccaaggacaccctcatgatctcccggacccctgaggtcacatgcgtggtggtggacgtgagccacgaagaccctgaggtcaagttcaactggtacgtggacggcgtggaggtgcataatgccaagacaaagccgcgggaggagcagtacaacagcacgtaccgtgtggtcagcgtcctcaccgtcctgcaccaggactggctgaatggcaaggagtacaagtgcaaggtctccaacaaagccctcccagcccccatcgagaaaaccatctccaaagccaaaggtgggacccgtggggtgcgagggccacatggacagaggccggctcggcccaccctctgccctgagagtgaccgctgtaccaacctctgtccctacagggcagccccgagaaccacaggtgtacaccctgcccccatcccgggatgagctgaccaagaaccaggtcagcctgacctgcctggtcaaaggcttctatcccagcgacatcgccgtggagtgggagagcaatgggcagccggagaacaactacaagaccacgcctcccgtgctggactccgacggctccttcttcctctacagcaagctcaccgtggacaagagcaggtggcagcaggggaacgtcttctcatgctccgtgatgcatgaggctctgcacaaccactacacgcagaagagcctctccctgtctccgggtaaa

SEQ ID NO: 74 - DNA, 2004 bp, Artificial
  1519gH20 IgG1 heavy chain (V + human gamma-1 constant) with signal sequence
atggaatggagctgggtctttctcttcttcctgtcagtaactacaggagtccattctgaggtaccacttgtggaaagcggaggaggtcttgtgcagcctggaggaagtttacgtctctcttgtgctgtgtctggcttcaccttctccaattacggaatggtctgggtcagacaagcacctggaaagggtcttgaatgggtggcctatattgactctgacggggacaacacctactatcgggattccgtgaaaggacgcttcacaatctcccgagataacgccaagagctcactgtacctgcagatgaatagcctgagagccgaggatactgccgtgtactattgcacaacgggaatcgttaggccttttctgtactggggacagggcaccttggttactgtctcgagcgcttctacaaagggcccatcggtcttccccctggcaccctcctccaagagcacctctgggggcacagcggccctgggctgcctggtcaaggactacttccccgaaccggtgacggtgtcgtggaactcaggcgccctgaccagcggcgtgcacaccttcccggctgtcctacagtcctcaggactctactccctcagcagcgtggtgaccgtgccctccagcagcttgggcacccagacctacatctgcaacgtgaatcacaagcccagcaacaccaaggtcgacaagaaagttggtgagaggccagcacagggagggagggtgtctgctggaagccaggctcagcgctcctgcctggacgcatcccggctatgcagccccagtccagggcagcaaggcaggccccgtctgcctcttcacccggaggcctctgcccgccccactcatgctcagggagagggtcttctggctttttccccaggctctgggcaggcacaggctaggtgcccctaacccaggccctgcacacaaaggggcaggtgctgggctcagacctgccaagagccatatccgggaggaccctgcccctgacctaagcccaccccaaaggccaaactctccactccctcagctcggacaccttctctcctcccagatctgagtaactcccaatcttctctctgcagagcccaaatcttgtgacaaaactcacacatgcccaccgtgcccaggtaagccagcccaggcctcgccctccagctcaaggcgggacaggtgccctagagtagcctgcatccagggacaggccccagccgggtgctgacacgtccacctccatctcttcctcagcacctgaactcctggggggaccgtcagtcttcctcttccccccaaaacccaaggacaccctcatgatctcccggacccctgaggtcacatgcgtggtggtggacgtgagccacgaagaccctgaggtcaagttcaactggtacgtggacggcgtggaggtgcataatgccaagacaaagccgcgggaggagcagtacaacagcacgtaccgtgtggtcagcgtcctcaccgtcctgcaccaggactggctgaatggcaaggagtacaagtgcaaggtctccaacaaagccctcccagcccccatcgagaaaaccatctccaaagccaaaggtgggacccgtggggtgcgagggccacatggacagaggccggctcggcccaccctctgccctgagagtgaccgctgtaccaacctctgtccctacagggcagccccgagaaccacaggtgtacaccctgcccccatcccgggatgagctgaccaagaaccaggtcagcctgacctgcctggtcaaaggcttctatcccagcgacatcgccgtggagtgggagagcaatgggcagccggagaacaactacaagaccacgcctcccgtgctggactccgacggctccttcttcctctacagcaagctcaccgtggacaagagcaggtggcagcaggggaacgtcttctcatgctccgtgatgcatgaggctctgcacaaccactacacgcagaagagcctctccctgtctccgggtaaa

SEQ ID NO: 75 - DNA, 657 bp, Artificial
  1519 gL20 light chain (V + constant, mammalian expression alternative)
gatatccagatgacccagagcccatctagcttatccgcttccgttggtgatcgcgtgacaattacgtgtaagagctcccaatctctcgtgggtgcaagtggcaagacctatctgtactggctctttcagaagcctggcaaggcaccaaaacggctgatctatctggtgtctacccttgactctgggataccgtcacgattttccggatctgggagcggaactgagttcacactcacgatttcatcgctgcaacccgaggactttgctacctactactgcctgcaaggcactcatttccctcacactttcggccaggggacaaaactcgaaatcaaacgtacggtagcggccccatctgtcttcatcttcccgccatctgatgagcagttgaaatctggaactgcctctgttgtgtgcctgctgaataacttctatcccagagaggccaaagtacagtggaaggtggataacgccctccaatcgggtaactcccaggagagtgtcacagagcaggacagcaaggacagcacctacagcctcagcagcaccctgacgctgagcaaagcagactacgagaaacacaaagtctacgcctgcgaagtcacccatcagggcctgagctcgcccgtcacaaagagcttcaacaggggagagtgt

SEQ ID NO: 76 - DNA, 684 bp, Artificial
  1519gH20 Fab' heavy chain (V + human gamma-1 CH1 + hinge, mammalian expression one base change from SEQ ID NO: 38)
gaggtaccacttgtggaaagcggaggaggtcttgtgcagcctggaggaagtttacgtctctcttgtgctgtgtctggcttcaccttctccaattacggaatggtctgggtcagacaagcacctggaaagggtcttgaatgggtggcctatattgactctgacggggacaacacctactatcgggattccgtgaaaggacgcttcacaatctcccgagataacgccaagagctcactgtacctgcagatgaatagcctgagagccgaggatactgccgtgtactattgcacaacgggaatcgttaggccttttctgtactggggacagggcaccttggttactgtctcgagcgcttctacaaagggcccatcggtcttccccctggcaccctcctccaagagcacctctgggggcacagcggccctgggctgcctggtcaaggactacttccccgaaccggtgacggtgtcgtggaactcaggcgccctgaccagcggcgtgcacaccttcccggctgtcctacagtcctcaggactctactccctcagcagcgtggtgaccgtgccctccagcagcttgggcacccagacctacatctgcaacgtgaatcacaagcccagcaacaccaaggtggacaagaaagttgagcccaaatcttgtgacaaaactcacacatgcgccgcg

SEQ ID NO: 77 - DNA, 741 bp, Artificial
  1519 gH20 Fab' heavy chain with signal sequence (mammalian expression one base changed from SEQ ID NO: 42)
atggaatggagctgggtctttctcttcttcctgtcagtaactacaggagtccattctgaggtaccacttgtggaaagcggaggaggtcttgtgcagcctggaggaagtttacgtctctcttgtgctgtgtctggcttcaccttctccaattacggaatggtctgggtcagacaagcacctggaaagggtcttgaatgggtggcctatattgactctgacggggacaacacctactatcgggattccgtgaaaggacgcttcacaatctcccgagataacgccaagagctcactgtacctgcagatgaatagcctgagagccgaggatactgccgtgtactattgcacaacgggaatcgttaggccttttctgtactggggacagggcaccttggttactgtctcgagcgcttctacaaagggcccatcggtcttccccctggcaccctcctccaagagcacctctgggggcacagcggccctgggctgcctggtcaaggactacttccccgaaccggtgacggtgtcgtggaactcaggcgccctgaccagcggcgtgcacaccttcccggctgtcctacagtcctcaggactctactccctcagcagcgtggtgaccgtgccctccagcagcttgggcacccagacctacatctgcaacgtgaatcacaagcccagcaacaccaaggtggacaagaaagttgagcccaaatcttgtgacaaaactcacacatgcgccgcg

SEQ ID NO: 78 - protein, 346 aa, Artificial
  1519gL20 FabFv light chain (alternative sequence to SEQ ID NO: 46)
DIQMTQSPSSLSASVGDRVTITCKSSQSLVGASGKTYLYWLFQKPGKAPKRLIYLVSTLDSGIPSRFSGSGSGTEFTLTISSLQPEDFATYYCLQGTHFPHTFGQGTKLEIKRTVAAPSVFIFPPSDEQLKSGTASVVCLLNNFYPREAKVQWKVDNALQSGNSQESVTEQDSKDSTYSLSSTLTLSKADYEKHKVYACEVTHQGLSSPVTKSFNRGECGGGGSGGGGSGGGGSDIQMTQSPSSVSASVGDRVTITCQSSPSVWSNFLSWYQQKPGKAPKLLIYEASKLTSGVPSRFSGSGSGTDFTLTISSLQPEDFATYYCGGGYSSISDTTFGCGTKVEIKRT

SEQ ID NO: 79 - DNA, 1038 bp, Artificial
  1519gL20 FabFv light chain (alternative sequence to SEQ ID NO: 47)
gacatccagatgacccagtccccctccagcctgtccgcctccgtgggcgacagagtgaccatcacatgcaagtcctcccagtccctggtcggagcctccggcaagacctacctgtactggctgttccagaagcccggcaaggcccccaagcggctgatctacctggtgtctaccctggactccggcatcccctcccggttctccggctctggctctggcaccgagttcaccctgaccatctccagcctgcagcccgaggacttcgccacctactactgtctgcaaggcacccacttcccccacaccttcggccagggcaccaagctggaaatcaagcggaccgtagcggccccatctgtcttcatcttcccgccatctgatgagcagttgaaatctggaactgcctctgttgtgtgcctgctgaataacttctatcccagagaggccaaagtacagtggaaggtggataacgccctccaatcgggtaactcccaggagagtgtcacagagcaggacagcaaggacagcacctacagcctcagcagcaccctgacgctgagcaaagcagactacgagaaacacaaagtctacgcctgcgaagtcacccatcagggcctgagctcgcccgtcacaaagagcttcaacaggggagagtgtggtggaggtggctctggcggtggtggctccggaggcggaggaagcgacatccagatgacccagagcccttcctctgtaagcgccagtgtcggagacagagtgactattacctgccaaagctccccttcagtctggtccaattttctatcctggtatcagcaaaagcccggaaaggctcctaaattgctgatctacgaagcaagcaaactcaccagcggcgtgcccagcaggttcagcggcagtgggtctggaactgactttaccctgacaatctcctcactccagcccgaggacttcgccacctattactgcggtggaggttacagtagcataagtgatacgacatttggatgcggcactaaagtggaaatcaagcgtacc

SEQ ID NO: 80 - DNA, 1071 bp, Artificial
  1519gH20 FabFv heavy chain (alternative sequence to SEQ ID NO: 51)
gaggtgcccctggtggaatctggcggcggactggtgcagcctggcggctccctgagactgtcttgcgccgtgtccggcttcaccttctccaactacggcatggtctgggtccgacaggctcctggcaagggactggaatgggtggcctacatcgactccgacggcgacaacacctactaccgggactccgtgaagggccggttcaccatctcccgggacaacgccaagtcctccctgtacctgcagatgaactccctgcgggccgaggacaccgccgtgtactactgcaccaccggcatcgtgcggccctttctgtactggggccagggcaccctggtcaccgtgtcctctgcttctacaaagggcccatcggtcttccccctggcaccctcctccaagagcacctctgggggcacagcggccctgggctgcctggtcaaggactacttccccgaaccggtgacggtgtcgtggaactcaggcgccctgaccagcggcgtgcacaccttcccggctgtcctacagtcctctggactctactccctcagcagcgtggtgaccgtgccctccagcagcttgggcacccagacctacatctgcaacgtgaatcacaagcccagcaacaccaaggtggacaagaaagttgagcccaaatcttgttccggaggtggcggttccggaggtggcggtacaggtggcggtgggtccgaagtccagctgcttgaatccggaggcggactcgtgcagcccggaggcagtcttcgcttgtcctgcgctgtatctggaatcgacctgagcaattacgccatcaactgggtgagacaggcacctgggaaatgcctcgaatggatcggcattatatgggctagtgggacgaccttttatgctacatgggcgaagggtagattcacaatctcacgggataatagtaagaacacagtgtacctgcagatgaactccctgcgagcagaggataccgccgtttactattgtgctcgcactgtcccaggttatagcactgcaccctactttgatctgtgggggcagggcactctggtcaccgtctcgtcc

SEQ ID NO: 81 - protein, 112 aa, Artificial
  Rat Ab 1548 VL region (alternative sequence to SEQ ID NO: 58)
DVVMTQTPLSLSVAIGQPASISSKSSQSLVGAGGKTYLYWLLQRSGQSPKRLIYLVSTLDSGIPDRFSGSGAETDFTLKIRRVEADDLGVYYCLQGTHFPHTFGAGTNLEIK

SEQ ID NO: 82 - DNA, 336 bp, Artificial
  Rat Ab 1548 VL region (alternative sequence to SEQ ID NO: 59)
gatgttgtgatgacccagactccactgtctttgtcggttgccattggacaaccagcctccatctcttctaagtcaagtcagagcctcgtaggtgctggtggaaagacatatttgtattggttattacagaggtccggccagtctccaaagcgactaatctatctggtgtccacactggactctggaattcctgataggttcagtggcagtggagcagagacagattttactcttaaaatccgcagagtggaagccgatgatttgggagtttattactgcttgcaaggtacacattttcctcacacgtttggagctgggaccaacctggaaataaaa

SEQ ID NO: 83 - protein, 116 aa, Artificial
  Rat Ab 1548 VH region (alternative sequence to SEQ ID NO: 60)
EVPLVESGGGSVQPGRSMKLSCVVSGFTFSNYGMVWVRQAPKKGLEWVAYIGSDGDNTYYRDSVKGRFTISRNNAKSTLYLQMDSLRSEDTATYYCTTGIVRPFLYWGQGVMVTVS

SEQ ID NO: 84 - DNA, 348 bp, Artificial
  Rat Ab 1548 VH region (alternative sequence to SEQ IS NO: 61)
gaggtgccgctggtggagtctgggggcggctcagtgcagcctgggaggtccatgaaactctcctgtgtagtctcaggattcactttcagtaactatggcatggtctgggtccgccaggctccaaagaagggtctggagtgggtcgcatatattggttctgatggtgataatacttactaccgagattccgtgaagggccgattcactatctccagaaataatgcaaaaagcaccctatatttgcaaatggacagtctgaggtctgaggacacggccacttattactgtacaacagggattgtccggccctttctctactggggccaaggagtcatggtcacagtctcg

SEQ ID NO: 85 - DNA, 1947 bp, Artificial
  1519gH20 IgG1 heavy chain (V + human gamma-1 constant with exons one base change to SEQ ID NO: 71)
gaggtaccacttgtggaaagcggaggaggtcttgtgcagcctggaggaagtttacgtctctcttgtgctgtgtctggcttcaccttctccaattacggaatggtctgggtcagacaagcacctggaaagggtcttgaatgggtggcctatattgactctgacggggacaacacctactatcgggattccgtgaaaggacgcttcacaatctcccgagataacgccaagagctcactgtacctgcagatgaatagcctgagagccgaggatactgccgtgtactattgcacaacgggaatcgttaggccttttctgtactggggacagggcaccttggttactgtctcgagcgcttctacaaagggcccatcggtcttccccctggcaccctcctccaagagcacctctgggggcacagcggccctgggctgcctggtcaaggactacttccccgaaccggtgacggtgtcgtggaactcaggcgccctgaccagcggcgtgcacaccttcccggctgtcctacagtcctcaggactctactccctcagcagcgtggtgaccgtgccctccagcagcttgggcacccagacctacatctgcaacgtgaatcacaagcccagcaacaccaaggtggacaagaaagttggtgagaggccagcacagggagggagggtgtctgctggaagccaggctcagcgctcctgcctggacgcatcccggctatgcagccccagtccagggcagcaaggcaggccccgtctgcctcttcacccggaggcctctgcccgccccactcatgctcagggagagggtcttctggctttttccccaggctctgggcaggcacaggctaggtgcccctaacccaggccctgcacacaaaggggcaggtgctgggctcagacctgccaagagccatatccgggaggaccctgcccctgacctaagcccaccccaaaggccaaactctccactccctcagctcggacaccttctctcctcccagatctgagtaactcccaatcttctctctgcagagcccaaatcttgtgacaaaactcacacatgcccaccgtgcccaggtaagccagcccaggcctcgccctccagctcaaggcgggacaggtgccctagagtagcctgcatccagggacaggccccagccgggtgctgacacgtccacctccatctcttcctcagcacctgaactcctggggggaccgtcagtcttcctcttccccccaaaacccaaggacaccctcatgatctcccggacccctgaggtcacatgcgtggtggtggacgtgagccacgaagaccctgaggtcaagttcaactggtacgtggacggcgtggaggtgcataatgccaagacaaagccgcgggaggagcagtacaacagcacgtaccgtgtggtcagcgtcctcaccgtcctgcaccaggactggctgaatggcaaggagtacaagtgcaaggtctccaacaaagccctcccagcccccatcgagaaaaccatctccaaagccaaaggtgggacccgtggggtgcgagggccacatggacagaggccggctcggcccaccctctgccctgagagtgaccgctgtaccaacctctgtccctacagggcagccccgagaaccacaggtgtacaccctgcccccatcccgggatgagctgaccaagaaccaggtcagcctgacctgcctggtcaaaggcttctatcccagcgacatcgccgtggagtgggagagcaatgggcagccggagaacaactacaagaccacgcctcccgtgctggactccgacggctccttcttcctctacagcaagctcaccgtggacaagagcaggtggcagcaggggaacgtcttctcatgctccgtgatgcatgaggctctgcacaaccactacacgcagaagagcctctccctgtctccgggtaaa

SEQ ID NO: 86 - DNA, 2004 bp, Artificial
  1519gH20 IgG1 heavy chain (V + human gamma-1 constant) with signal sequence (one base change from SEQ ID NO:72)
atggaatggagctgggtctttctcttcttcctgtcagtaactacaggagtccattctgaggtaccacttgtggaaagcggaggaggtcttgtgcagcctggaggaagtttacgtctctcttgtgctgtgtctggcttcaccttctccaattacggaatggtctgggtcagacaagcacctggaaagggtcttgaatgggtggcctatattgactctgacggggacaacacctactatcgggattccgtgaaaggacgcttcacaatctcccgagataacgccaagagctcactgtacctgcagatgaatagcctgagagccgaggatactgccgtgtactattgcacaacgggaatcgttaggccttttctgtactggggacagggcaccttggttactgtctcgagcgcttctacaaagggcccatcggtcttccccctggcaccctcctccaagagcacctctgggggcacagcggccctgggctgcctggtcaaggactacttccccgaaccggtgacggtgtcgtggaactcaggcgccctgaccagcggcgtgcacaccttcccggctgtcctacagtcctcaggactctactccctcagcagcgtggtgaccgtgccctccagcagcttgggcacccagacctacatctgcaacgtgaatcacaagcccagcaacaccaaggtggacaagaaagttggtgagaggccagcacagggagggagggtgtctgctggaagccaggctcagcgctcctgcctggacgcatcccggctatgcagccccagtccagggcagcaaggcaggccccgtctgcctcttcacccggaggcctctgcccgccccactcatgctcagggagagggtcttctggctttttccccaggctctgggcaggcacaggctaggtgcccctaacccaggccctgcacacaaaggggcaggtgctgggctcagacctgccaagagccatatccgggaggaccctgcccctgacctaagcccaccccaaaggccaaactctccactccctcagctcggacaccttctctcctcccagatctgagtaactcccaatcttctctctgcagagcccaaatcttgtgacaaaactcacacatgcccaccgtgcccaggtaagccagcccaggcctcgccctccagctcaaggcgggacaggtgccctagagtagcctgcatccagggacaggccccagccgggtgctgacacgtccacctccatctcttcctcagcacctgaactcctggggggaccgtcagtcttcctcttccccccaaaacccaaggacaccctcatgatctcccggacccctgaggtcacatgcgtggtggtggacgtgagccacgaagaccctgaggtcaagttcaactggtacgtggacggcgtggaggtgcataatgccaagacaaagccgcgggaggagcagtacaacagcacgtaccgtgtggtcagcgtcctcaccgtcctgcaccaggactggctgaatggcaaggagtacaagtgcaaggtctccaacaaagccctcccagcccccatcgagaaaaccatctccaaagccaaaggtgggacccgtggggtgcgagggccacatggacagaggccggctcggcccaccctctgccctgagagtgaccgctgtaccaacctctgtccctacagggcagccccgagaaccacaggtgtacaccctgcccccatcccgggatgagctgaccaagaaccaggtcagcctgacctgcctggtcaaaggcttctatcccagcgacatcgccgtggagtgggagagcaatgggcagccggagaacaactacaagaccacgcctcccgtgctggactccgacggctccttcttcctctacagcaagctcaccgtggacaagagcaggtggcagcaggggaacgtcttctcatgctccgtgatgcatgaggctctgcacaaccactacacgcagaagagcctctccctgtctccgggtaaa

SEQ ID NO: 87 - protein, 444 aa, Artificial
  1519gH20 IgG4 heavy chain (V + human gamma-4 constant no P mutations)
EVPLVESGGGLVQPGGSLRLSCAVSGFTFSNYGMVWVRQAPGKGLEWVAYIDSDGDNTYYRDSVKGRFTISRDNAKSSLYLQMNSLRAEDTAVYYCTTGIVRPFLYWGQGTLVTVSSASTKGPSVFPLAPCSRSTSESTAALGCLVKDYFPEPVTVSWNSGALTSGVHTFPAVLQSSGLYSLSSVVTVPSSSLGTKTYTCNVDHKPSNTKVDKRVESKYGPPCPSCPAPEFLGGPSVFLFPPKPKDTLMISRTPEVTCVVVDVSQEDPEVQFNWYVDGVEVHNAKTKPREEQFNSTYRVVSVLTVLHQDWLNGKEYKCKVSNKGLPSSIEKTISKAKGQPREPQVYTLPPSQEEMTKNQVSLTCLVKGFYPSDIAVEWESNGQPENNYKTTPPVLDSDGSFFLYSRLTVDKSRWQEGNVFSCSVMHEALHNHYTQKSLSLSLGK

SEQ ID NO: 88 - DNA, 1939 bp, Artificial
  1519gH20 IgG4 heavy chain (V + human gamma-4 constant with exons no P mutations)
gaggtaccacttgtggaaagcggaggaggtcttgtgcagcctggaggaagtttacgtctctcttgtgctgtgtctggcttcaccttctccaattacggaatggtctgggtcagacaagcacctggaaagggtcttgaatgggtggcctatattgactctgacggggacaacacctactatcgggattccgtgaaaggacgcttcacaatctcccgagataacgccaagagctcactgtacctgcagatgaatagcctgagagccgaggatactgccgtgtactattgcacaacgggaatcgttaggccttttctgtactggggacagggcaccttggttactgtctcgagcgcttctacaaagggcccatccgtcttccccctggcgccctgctccaggagcacctccgagagcacagccgccctgggctgcctggtcaaggactacttccccgaaccggtgacggtgtcgtggaactcaggcgccctgaccagcggcgtgcacaccttcccggctgtcctacagtcctcaggactctactccctcagcagcgtggtgaccgtgccctccagcagcttgggcacgaagacctacacctgcaacgtagatcacaagcccagcaacaccaaggtggacaagagagttggtgagaggccagcacagggagggagggtgtctgctggaagccaggctcagccctcctgcctggacgcaccccggctgtgcagccccagcccagggcagcaaggcatgccccatctgtctcctcacccggaggcctctgaccaccccactcatgcccagggagagggtcttctggatttttccaccaggctccgggcagccacaggctggatgcccctaccccaggccctgcgcatacaggggcaggtgctgcgctcagacctgccaagagccatatccgggaggaccctgcccctgacctaagcccaccccaaaggccaaactctccactccctcagctcagacaccttctctcctcccagatctgagtaactcccaatcttctctctgcagagtccaaatatggtcccccatgcccatcatgcccaggtaagccaacccaggcctcgccctccagctcaaggcgggacaggtgccctagagtagcctgcatccagggacaggccccagccgggtgctgacgcatccacctccatctcttcctcagcacctgagttcctggggggaccatcagtcttcctgttccccccaaaacccaaggacactctcatgatctcccggacccctgaggtcacgtgcgtggtggtggacgtgagccaggaagaccccgaggtccagttcaactggtacgtggatggcgtggaggtgcataatgccaagacaaagccgcgggaggagcagttcaacagcacgtaccgtgtggtcagcgtcctcaccgtcctgcaccaggactggctgaacggcaaggagtacaagtgcaaggtctccaacaaaggcctcccgtcctccatcgagaaaaccatctccaaagccaaaggtgggacccacggggtgcgagggccacatggacagaggtcagctcggcccaccctctgccctgggagtgaccgctgtgccaacctctgtccctacagggcagccccgagagccacaggtgtacaccctgcccccatcccaggaggagatgaccaagaaccaggtcagcctgacctgcctggtcaaaggcttctaccccagcgacatcgccgtggagtgggagagcaatgggcagccggagaacaactacaagaccacgcctcccgtgctggactccgacggctccttcttcctctacagcaggctaaccgtggacaagagcaggtggcaggaggggaatgtcttctcatgctccgtgatgcatgaggctctgcacaaccactacacacagaagagcctctccctgtctctgggtaaa

SEQ ID NO: 89 - DNA, 1996 bp, Artificial
  1519gH20 IgG4 heavy chain (V + human gamma-4 constant) with signal sequence - no P mutation
atggaatggagctgggtctttctcttcttcctgtcagtaactacaggagtccattctgaggtaccacttgtggaaagcggaggaggtcttgtgcagcctggaggaagtttacgtctctcttgtgctgtgtctggcttcaccttctccaattacggaatggtctgggtcagacaagcacctggaaagggtcttgaatgggtggcctatattgactctgacggggacaacacctactatcgggattccgtgaaaggacgcttcacaatctcccgagataacgccaagagctcactgtacctgcagatgaatagcctgagagccgaggatactgccgtgtactattgcacaacgggaatcgttaggccttttctgtactggggacagggcaccttggttactgtctcgagcgcttctacaaagggcccatccgtcttccccctggcgccctgctccaggagcacctccgagagcacagccgccctgggctgcctggtcaaggactacttccccgaaccggtgacggtgtcgtggaactcaggcgccctgaccagcggcgtgcacaccttcccggctgtcctacagtcctcaggactctactccctcagcagcgtggtgaccgtgccctccagcagcttgggcacgaagacctacacctgcaacgtagatcacaagcccagcaacaccaaggtggacaagagagttggtgagaggccagcacagggagggagggtgtctgctggaagccaggctcagccctcctgcctggacgcaccccggctgtgcagccccagcccagggcagcaaggcatgccccatctgtctcctcacccggaggcctctgaccaccccactcatgcccagggagagggtcttctggatttttccaccaggctccgggcagccacaggctggatgcccctaccccaggccctgcgcatacaggggcaggtgctgcgctcagacctgccaagagccatatccgggaggaccctgcccctgacctaagcccaccccaaaggccaaactctccactccctcagctcagacaccttctctcctcccagatctgagtaactcccaatcttctctctgcagagtccaaatatggtcccccatgcccatcatgcccaggtaagccaacccaggcctcgccctccagctcaaggcgggacaggtgccctagagtagcctgcatccagggacaggccccagccgggtgctgacgcatccacctccatctcttcctcagcacctgagttcctggggggaccatcagtcttcctgttccccccaaaacccaaggacactctcatgatctcccggacccctgaggtcacgtgcgtggtggtggacgtgagccaggaagaccccgaggtccagttcaactggtacgtggatggcgtggaggtgcataatgccaagacaaagccgcgggaggagcagttcaacagcacgtaccgtgtggtcagcgtcctcaccgtcctgcaccaggactggctgaacggcaaggagtacaagtgcaaggtctccaacaaaggcctcccgtcctccatcgagaaaaccatctccaaagccaaaggtgggacccacggggtgcgagggccacatggacagaggtcagctcggcccaccctctgccctgggagtgaccgctgtgccaacctctgtccctacagggcagccccgagagccacaggtgtacaccctgcccccatcccaggaggagatgaccaagaaccaggtcagcctgacctgcctggtcaaaggcttctaccccagcgacatcgccgtggagtgggagagcaatgggcagccggagaacaactacaagaccacgcctcccgtgctggactccgacggctccttcttcctctacagcaggctaaccgtggacaagagcaggtggcaggaggggaatgtcttctcatgctccgtgatgcatgaggctctgcacaaccactacacacagaagagcctctccctgtctctgggtaaa

SEQ ID NO: 90 - DNA, 336 bp, Artificial
  1519 gL20 V-region (mammalian expression alternative to SEQ ID NO: 17)
gacatccagatgacccagtccccctccagcctgtccgcctccgtgggcgacagagtgaccatcacatgcaagtcctcccagtccctggtcggagcctccggcaagacctacctgtactggctgttccagaagcccggcaaggcccccaagcggctgatctacctggtgtctaccctggactccggcatcccctcccggttctccggctctggctctggcaccgagttcaccctgaccatctccagcctgcagcccgaggacttcgccacctactactgtctgcaaggcacccacttcccccacaccttcggccagggcaccaagctggaaatcaag

SEQ ID NO: 91 - DNA, 657 bp, Artificial
  1519 gL20 light chain (V + constant, mammalian expression) alternative to SEQ ID NO: 24)
gacatccagatgacccagtccccctccagcctgtccgcctccgtgggcgacagagtgaccatcacatgcaagtcctcccagtccctggtcggagcctccggcaagacctacctgtactggctgttccagaagcccggcaaggcccccaagcggctgatctacctggtgtctaccctggactccggcatcccctcccggttctccggctctggctctggcaccgagttcaccctgaccatctccagcctgcagcccgaggacttcgccacctactactgtctgcaaggcacccacttcccccacaccttcggccagggcaccaagctggaaatcaagcggaccgtggccgctccctccgtgttcatcttcccaccctccgacgagcagctgaagtccggcaccgcctccgtcgtgtgcctgctgaacaacttctacccccgcgaggccaaggtgcagtggaaggtggacaacgccctgcagtccggcaactcccaggaatccgtcaccgagcaggactccaaggacagcacctactccctgtcctccaccctgaccctgtccaaggccgactacgagaagcacaaggtgtacgcctgcgaagtgacccaccagggcctgtccagccccgtgaccaagtccttcaaccggggcgagtgc

SEQ ID NO: 92 - DNA, 348 bp, Artificial
  1519 gH20 V-region (mammalian expression alternative to SEQ ID NO: 31)
gaggtgcccctggtggaatctggcggcggactggtgcagcctggcggctccctgagactgtcttgcgccgtgtccggcttcaccttctccaactacggcatggtctgggtccgacaggctcctggcaagggactggaatgggtggcctacatcgactccgacggcgacaacacctactaccgggactccgtgaagggccggttcaccatctcccgggacaacgccaagtcctccctgtacctgcagatgaactccctgcgggccgaggacaccgccgtgtactactgcaccaccggcatcgtgcggccctttctgtactggggccagggcaccctggtcaccgtgtcc

SEQ ID NO: 93 - DNA, 1332 bp, Artificial
  1519gH20 IgG4 heavy chain (V + human gamma-4P constant alternative to SEQ ID NO: 44)
gaggtgcccctggtggaatctggcggcggactggtgcagcctggcggctccctgagactgtcttgcgccgtgtccggcttcaccttctccaactacggcatggtctgggtccgacaggctcctggcaagggactggaatgggtggcctacatcgactccgacggcgacaacacctactaccgggactccgtgaagggccggttcaccatctcccgggacaacgccaagtcctccctgtacctgcagatgaactccctgcgggccgaggacaccgccgtgtactactgcaccaccggcatcgtgcggccctttctgtactggggccagggcaccctggtcaccgtgtcctctgcctccaccaagggcccctccgtgttccctctggccccttgctcccggtccacctccgagtctaccgccgctctgggctgcctggtcaaggactacttccccgagcccgtgacagtgtcctggaactctggcgccctgacctccggcgtgcacaccttccctgccgtgctgcagtcctccggcctgtactccctgtcctccgtcgtgaccgtgccctcctccagcctgggcaccaagacctacacctgtaacgtggaccacaagccctccaacaccaaggtggacaagcgggtggaatctaagtacggccctccctgccccccctgccctgcccctgaatttctgggcggaccttccgtgttcctgttccccccaaagcccaaggacaccctgatgatctcccggacccccgaagtgacctgcgtggtggtggacgtgtcccaggaagatcccgaggtccagttcaattggtacgtggacggcgtggaagtgcacaatgccaagaccaagcccagagaggaacagttcaactccacctaccgggtggtgtccgtgctgaccgtgctgcaccaggactggctgaacggcaaagagtacaagtgcaaggtgtccaacaagggcctgccctccagcatcgaaaagaccatctccaaggccaagggccagccccgcgagccccaggtgtacaccctgccccctagccaggaagagatgaccaagaaccaggtgtccctgacctgtctggtcaagggcttctacccctccgacattgccgtggaatgggagtccaacggccagcccgagaacaactacaagaccaccccccctgtgctggacagcgacggctccttcttcctgtactctcggctgaccgtggacaagtcccggtggcaggaaggcaacgtcttctcctgctccgtgatgcacgaggccctgcacaaccactacacccagaagtccctgtccctgagcctgggcaag

SEQ ID NO: 94 - protein, 274 aa, Artificial
  FcRn alpha chain extracellular sequence
AESHLSLLYHLTAVSSPAPGTPAFWVSGWLGPQQYLSYNSLRGEAEPCGAWVWENQVSWYWEKETTDLRIKEKLFLEAFKALGGKGPYTLQGLLGCELGPDNTSVPTAKFALNGEEFMNFDLKQGTWGGDWPEALAISQRWQQQDKAANKELTFLLFSCPHRLREHLERGRGNLEWKEPPSMRLKARPSSPGFSVLTCSAFSFYPPELQLRFLRNGLAAGTGQGDFGPNSDGSFHASSSLTVKSGDEHHYCCIVQHAGLAQPLRVELESPAKSS

SEQ ID NO: 95 - protein, 99 aa, Homo sapiens
IQKTPQIQVYSRHPPENGKPNFLNCYVSQFHPPQIEIELLKNGKKIPNIEMSDLSFSKDWSFYILAHTEFTPTETDVYACRVKHVTLKEPKTVTWDRDM